European Patent Specification EP 3 678 673 B1, published January 25, 2023. Title: COMPOSITIONS AND PROCESSES FOR TARGETED DELIVERY, EXPRESSION AND MODULATION OF CODING RIBONUCLEIC ACIDS IN TISSUE. Applicant: Combined Therapeutics. The sequence listing filed with the application follows.

SEQUENCE LISTING (5 sequences)

SEQ ID NO: 1 - RNA, 22 nt, Artificial Sequence
  single miR122 binding site
aacgccauuaucacacuaaaua

SEQ ID NO: 2 - RNA, 50 nt, Artificial Sequence
  2x miR-122 binding sites with linker
aacgccauuaucacacuaaauauuuaaaaacgccauuaucacacuaaaua

SEQ ID NO: 3 - RNA, 761 nt, Artificial Sequence
  mCherry sequence with 2x miR-122 binding sequence and linker
auggugagcaagggcgaggaggauaacauggccaucaucaaggaguucaugcgcuucaaggugcacauggagggcuccgugaacggccacgaguucgagaucgagggcgagggcgagggccgccccuacgagggcacccagaccgccaagcugaaggugaccaaggguggcccccugcccuucgccugggacauccuguccccucaguucauguacggcuccaaggccuacgugaagcaccccgccgacauccccgacuacuugaagcuguccuuccccgagggcuucaagugggagcgcgugaugaacuucgaggacggcggcguggugaccgugacccaggacuccucccugcaggacggcgaguucaucuacaaggugaagcugcgcggcaccaacuuccccuccgacggccccguaaugcagaagaagaccaugggcugggaggccuccuccgagcggauguaccccgaggacggcgcccugaagggcgagaucaagcagaggcugaagcugaaggacggcggccacuacgacgcugaggucaagaccaccuacaaggccaagaagcccgugcagcugcccggcgccuacaacgucaacaucaaguuggacaucaccucccacaacgaggacuacaccaucguggaacaguacgaacgcgccgagggccgccacuccaccggcggcauggacgagcuguacaaguaaaacgccauuaucacacuaaauauuuaaaaacgccauuaucacacuaaaua

SEQ ID NO: 4 - RNA, 1496 nt, Artificial Sequence
  US3 with 2x miR-122 binding sites and linker
auggccugucguaaguuuugucgcguuuacgggggacagggcaggaggaaggaggaggccgucccgccggagacaaagccgucccggguguuuccucauggccccuuuuauaccccagccgaggacgcgugccuggacuccccgcccccggagacccccaaaccuucccacaccacaccacccggcgaugccgagcgccugugucaucugcaggagauccuggcccagauguacggaaaccaggacuaccccauagaggacgaccccagcgcggaugccgcggacgaugucgacgaggacgccccggacgacguggccuauccggaggaauacgcagaggagcuuuuucugcccggggacgcgcccgguccccuuaucggggccaacgaccacaucccucccccguguggcgcaucuccccccgguauacgacgacgcagccgggaugagauuggggccacgggauuuaccgcggaagaacuggacgccauggacagggaggcggcucgagccaucagccgcggcggcaagccccccucgaccauggccaagcuggugacuggcaugggcuuuacgauccacggagcgcucaccccaggaucggaggggugugucuuugacagcagccacccagauuacccccaacggguaaucgugaaggcggggugguacacgagcacgagccacgaggcgcgacugcugaggcgacuggaccaccccgcgauccugccccuccuggaccugcaugucgucuccggggucacgugucugguccuccccaaguaccaggccgaccuguauaccuaucugaguaggcgccugaacccgcugggacgcccgcagaucgcagcggucucccggcagcuccuaagcgccguugacuacauucaccgccagggcauuauccaccgcgacauuaagaccgaaaauauuuuuauuaacacccccgaggacauuugccugggggacuuuggugccgcgugcuucgugcaggguucccgaucaagccccuuccccuacggaaucgccggaaccaucgacaccaacgcccccgagguccugaccggggauccguauaccaccaccgucgacauuuggagcgccggucuggugaucuucgagacugccguccacaacgcguccuuguucucggccccccgcggccccaaaaggggcccgugcgacagucagaucacccgcaucauccgacaggcccagguccacguugacgaguuuuccccgcauccagaaucgcgccucaccucgcgcuaccgcucccgcgcggccgggaacaaucgcccgccguacacccgaccggccuggacccgcuacuacaagauggacauagacgucgaauaucugguuugcaaagcccucaccuucgacggcgcgcuucgccccagcgccgcagagcugcuuuguuugccgcuguuucaacagaaaugaaacgccauuaucacacuaaauauuuaaaaacgccauuaucacacuaaaua

SEQ ID NO: 5 - RNA, 3466 nt, Artificial Sequence
  ICP6 with 2x miRNA-122 binding site sequences
augauggccagccgcccagccgcauccucucccgucgaagcgcgggccccgguugggggacaggaggccggcggccccagcgcagccacccagggggaggccgccggggccccucucgcccacggccaccacguguacugccagcgagucaauggcgugauggugcuuuccgacaagacgcccggguccgcguccuaccgcaucagcgauagcaacuuuguccaaugugguuccaacugcaccaugauuaucgacggagacguggugcgcgggcgcccccaggacccgggggccgcggcaucccccgcucccuucguugcggugacaaacaucggagccggcagcgacggcgggaccgccgucguugcauucgggggaaccccacgucgcucggcggggacgucuaccgguacccagacggccgacgucccagccgaggcccuugggggccccccuccuccuccccgcuucacccuggguggcggcuguugcuccugucgcgacacacggcgccgcucugcgguauucgggggggagggggaucccgucggccccgcggaguucgucucggacgaccggucguccgauuccgacucggaugacucggaggacaccgacucggagacgcugucacacgccuccucggacguguccggcggggccacguacgacgacgcccuugacuccgauucgucaucggaugacucccugcagauagauggccccgugugucgcccguggagcaaugacaccgcgccccuggauguuugccccgggacccccggcccgggcgccgacgccgguggucccucagcgguagacccacacgcgccgacgacaggggccggcgcuggucuugcggccgaucccgccguggcccgggacgacgcggaggggcuuucggacccccggccacgucugggaacgggcacggccuaccccgucccccuggaacucacgcccgagaacgcggaggccguggcgcgcuuucugggagaugccgugaaccgcgaacccgcgcucaugcuggaguacuuuugccggugcgcccgcgaggaaaccaagcgugucccccccaggacauucugcagccccccucgccucacggaggacgacuuugggcuucucaacuacgcgcucguggagaugcagcgccugugucuggacguuccuccggucccgccgaacgcauacaugcccuauuaucucagggaguaugugacgcggcuggucaacggguucaagccgcuggugagccgguccguucgccuuuaccgcauccuggggguucuggugcaccugcggauccggacccgggaggccuccuuugaggaguggcugcgauccaaggaaguggcccuggacuuuggccugacggaaaggcuucgcgagcacgaagcccagcuggugauccuggcccaggcucuggaccauuacgacugucugauccacagcacaccgcacacgcuggucgagcgggggcugcaaucggcccugaaguaugaggaguuuuaccuaaagcgcuuuggcgggcacuacauggaguccgucuuccagauguacacccgcaucgccggcuuuuuggccugccgggccacgcgcggcaugcgccacaucgcccuggggcgagaggggucguggugggaaauguucaaguucuuuuuccaccgccucuacgaccaccagaucguaccgucgacccccgccaugcugaaccuggggacccgcaacuacuacaccuccagcugcuaccugguaaacccccaggccaccacaaacaaggcgacccugcgggccaucaccagcaacgucagugccauccucgcccgcaacgggggcaucgggcuaugcgugcaggcguuuaacgacuccggccccgggaccgccagcgucaugcccgcccucaagguccucgacucgcugguggcggcgcacaacaaagagagcgcgcguccgaccggcgcgugcguguaccuggagccguggcacaccgacgugcgggccgugcuccggaugaaggggguccucgccggcgaagaggcccagcgcugcgacaauaucuucagcgcccucuggaugccagaccuguuuuucaagcgccugauucgccaccuggacggcgagaagaacgucacauggacccuguucgaccgggacaccagcaugucgcucgccgacuuucacggggaggaguucgagaagcucuaccagcaccucgaggucaugggguucggcgagcagauacccauccaggagcuggccuauggcauugugcgcagugcggccacgaccgggagccccuucgucauguucaaagacgcggugaaccgccacuacaucuacgacacccagggggcggccaucgccggcuccaaccucugcaccgagaucguccauccggccuccaagcgauccaguggggucugcaaucugggaagcgugaaucuggcccgaugcgucuccaggcagacguuugacuuugggcggcuccgcgacgccgugcaggcgugcgugcugauggugaacaucaugaucgacagcacgcuacaacccacgccccagugcacccgcggcaacgacaaccugcgguccaugggaaucggcaugcagggccugcacacggccugccugaagcuggggcuggaucuggagucugccgaauuucaggaccugaacaaacacaucgccgaggugaugcugcugucggcgaugaagaccagcaacgcgcugugcguucgcggggcccgucccuucaaccacuuuaagcgcagcauguaucgcgccggccgcuuucacugggagcgcuuuccggacgcccggccgcgguacgagggcgagugggagaugcuacgccagagcaugaugaaacacggccugcgcaacagccaguuugucgcgcugaugcccaccgccgccucggcgcagaucucggacgucagcgagggcuuugccccccuguucaccaaccuguuuagcaaggugacccgggacggcgagacgcugcgccccaacacgcuccugcuaaaggaacuggaacgcacguuuagcgggaagcgccuccuggaggugauggacaguucgacgccaagcagugguccguggcgcaggcgcucccgugccuggagcccacccacccccuccggcgauucaagaccgcguuugacuacgaccagaaguugcugaucgaccugugugcggaccgcgcccccuacgucgaccauagccaauccaugacccuguaugucacggagaaggcggacgggacccucccagccuccacccugguccgccuucugguccacgcauauaagcgcggacuaaaaacagggauguacuacugcaagguucgcaaggcgaccaacagcggggucuuuggcggcgacgacaacauugucugcacgagcugcgcgcuguagaacgccauuaucacacuaaauauuuaaaaacgccauuaucacacuaaaua